European Patent Application EP 4 257 693 A1, published October 11, 2023. Title: SACCHAROMYCES CEREVISIAE MUTANT STRAIN FOR PRODUCING SPHINGOSINE AND SPHINGOSINE 1-PHOSPHATE AND METHOD FOR PRODUCING THE SAME. Applicant: KOREA INSTITUTE OF INDUSTRIAL TECHNOLOGY. The sequence listing filed with the application follows.

SEQUENCE LISTING (4 sequences)

SEQ ID NO: 1 - DNA, 969 bp, Artificial
  hDES1
atgggcagtagagtcagtagagaagactttgaatgggtctatacggatcagccgcatgctgacaggagaagggaaatattggcaaagtatccagaaatcaagtcattgatgaagcccgaccctaacctaatctggataataataatgatggtacttacccaacttggtgcattttacattgtaaaggatctagattggaagtgggtaatctttggtgcatacgcctttgggtcatgtatcaaccacagtatgaccctagcgattcatgaaatcgcccacaacgcagcatttgggaattgtaaggcgatgtggaacaggtggtttggcatgtttgctaacttgccaatcggaataccgtactctattagtttcaaacgttatcacatggatcaccatcgttatctgggggctgacggtgttgatgtagacataccgaccgacttcgaaggatggttcttctgtactgcctttagaaagtttatctgggtgattctgcaaccactattttatgcgttcagaccgctgtttataaatcccaaaccgatcacatacttagaggttataaacactgtagcgcaagttacttttgacatactaatctattattttttgggcataaagtctctagtgtatatgcttgcagcttctttattggggttgggtctgcacccaatcagcggacacttcatagccgaacactacatgtttttaaaaggacacgaaacgtactcttattatggtccgctgaatttacttacattcaacgtaggctatcataacgaacaccacgattttccgaatatcccagggaagagccttccactggttagaaaaattgcagcggagtactacgataatcttccacattacaactcttggatcaaggttctatacgattttgtgatggacgatacaattagcccatactccaggatgaaacgtcaccagaagggggagatggttttagag

SEQ ID NO: 2 - DNA, 792 bp, Artificial
  ACER1
atgccaagtatcttcgcgtaccagtcaagtgaagtggattggtgtgagtcaaattttcagtactcagagcttgttgcggagttttacaatacgttttcaaacataccattctttatattcggcccacttatgatgttgttaatgcatccttacgcacagaagagaagcagatatatatacgttgtttgggttctttttatgataatagggctgtttagtatgtatttccacatgactctgtcctttctgggtcaactactagacgagatagcgatcctatggctattagggtccggatattccatctggatgccccgttgctattttccatcattcctgggcggtaacaggtctcagtttataagattagtgtttatcacgactgtggttagcactttgctttccttccttagacccaccgtaaatgcatacgctttgaatagtatagcgctgcacatcttgtatatagtatgccaggagtacaggaaaacttcaaataaggaattgaggcatttgatagaagtatcagtagtactttgggcggtggccttgacatcttggatcagtgatagacttctttgcagtttttggcaaaggattcattttttctaccttcactctatatggcacgtgctgataagtatcacgttcccttacggtatggtgacaatggcattagtagacgccaactatgaaatgcccggcgagacactgaaagtaagatactggccgagagattcatggccagtaggtctaccctatgttgagataaggggagatgataaagactgt

SEQ ID NO: 3 - DNA, 1881 bp, Artificial
  SMPD1
atgcctagatatggtgcttccttacgtcagagttgtccaaggagtggcagggaacaagggcaggacggaactgccggagccccaggactgctgtggatgggtttagctctagctttagctttggctttagcactatctgactctagggtcttgtgggcgccggcagaagcgcatccgctttcccctcaagggcacccagcccgtttacacagaatagttccacgtctaagggacgtcttcggctggggaaacctgacgtgccctatctgtaaaggattattcacagcgattaatctaggactaaagaaggaacctaacgtggcgagagtggggagcgtagcaatcaaactgtgtaacttgctaaaaattgctcctcccgctgtctgccagtccatcgtccacttgttcgaagatgatatggtggaggtctggagaagaagtgttctttcaccgagcgaggccagaggtcttctgcttgggagtacctgtggtcattgggacatcttttctagttggaacatctctctaccgactgtgccaaagccgccccctaaaccccctagtccgccagcacccggggcccccgtcagtagaatattattcctgacggaccttcattgggaccacgattatttagaaggaacggacccggactgtgcggacccgctttgttgcagacgtggttctggcctgccgcccgcctcccgtccgggtgcggggtactggggtgaatacagcaagtgtgacctgcccctgagaacgcttgagtcactgctttccggccttggcccggccggaccctttgacatggtgtactggactggtgatatccctgcacatgatgtctggcatcaaactcgtcaggaccagcttagagcattaactactgtgacagcgctagttagaaaatttttgggcccggtgcccgtatatccggccgtaggtaatcatgaaagtacccccgtaaactcttttccccctccgtttattgaaggaaatcacagctcaagatggttatatgaagcgatggcaaaggcgtgggagccatggcttcccgccgaagcgctaaggactctgaggattggtgggttctatgccctaagtccgtacccagggttgagattaatctccttgaatatgaatttctgctctagagagaacttttggttacttatcaatagcactgatccggccggtcaactacagtggttagtgggggagttacaggcggcggaagaccgtggagacaaagtacatatcatcggacacataccacctggacattgtttaaagagctggtcatggaattactataggatagttgccagatatgaaaatacgctagccgcccagttttttggacatactcatgtcgatgaatttgaagttttctatgatgaagagactctgagtagaccactggcggtcgcattcttggcgcctagcgcaaccacgtacatagggttgaacccaggctatcgtgtttaccagatagatggaaactattcaggcagctcccatgtcgtactggaccatgaaacttatatactgaatctgacccaagccaacataccgggtgccattccgcattggcagcttctttatagagcccgtgagacttatggattaccaaacaccctaccaacggcctggcataacctagtgtataggatgcgtggggacatgcaattatttcagacgttttggttcctgtatcacaagggtcatccacccagtgaaccttgcggtacaccttgcagattggcgaccctttgcgcgcagttatcagcgcgtgcggacagcccagcgttgtgcaggcacctgatgccggatgggtctcttcctgaagcgcaaagcctttggcccaggcccttgttttgt

SEQ ID NO: 4 - DNA, 1152 bp, Artificial
  hSPHK1
atggatcctgctggaggtccgaggggggttttgccccgtccatgccgtgtgttagttttacttaatcccaggggtggcaaaggcaaggcgttgcagttattcaggagtcacgtccagcccttgttggccgaagctgagatttctttcacactaatgcttacggaaaggcgtaaccatgcgagggaactggttcgttccgaagaacttgggcgttgggatgcattggtagtaatgtcaggcgacggacttatgcatgaagtggtcaatgggctgatggaaagaccggactgggagactgccattcaaaaaccgctatgctccttacccgccgggtctggaaacgcattagccgcgagccttaaccactacgccgggtacgagcaagtcacaaacgaagatcttctaacaaactgcacgttacttctttgccgtagactgctatccccgatgaatttactttccctgcatacagccagcggattaagacttttttctgtgcttagtttggcgtggggctttatagcggacgttgatcttgaatccgaaaaatacagaagattaggtgagatgagatttacgttaggtacattcctaaggttagctgcgttaagaacatatagaggtaggctggcttatttgccggttggtcgtgtgggtagcaagaccccggcgagtccagtagtagtccagcaaggccctgtcgatgcccacttagtaccgctggaagagccggttccgtctcattggacggtcgttcctgacgaggattttgtcttagttcttgcccttctgcactcccaccttgggtccgaaatgtttgcagctcctatggggcgttgcgctgccggagtaatgcatttgttctacgtaagggctggggtcagcagagcaatgttgctacgtttatttcttgcaatggagaaaggaagacatatggagtatgaatgtccatatcttgtgtatgtgccggttgttgcattccgtttagagccaaaagacggtaagggcgtcttcgctgtcgatggtgaactaatggtctccgaggcagtgcaaggtcaggttcatccgaattatttctggatggtgagtggctgtgtggaaccccctcctagctggaaacctcagcaaatgcctccgcccgaggaacctcta